European Patent Specification EP 4 558 516 B1, published August 13, 2025. Title: ALBUMIN PROTEIN VARIANTS, PRODUCTION THEREOF AND USES OF SAME. Applicant: Yeda Research and Development Co. Ltd. The sequence listing filed with the application follows.

SEQUENCE LISTING (18 sequences)

SEQ ID NO: 1 - protein, 586 aa, Homo sapiens
  source 1..586: note = Amino Acid sequence of mature HSA
MDAHKSEVAHRFKDLGEENFKALVLIAFAQYLQQCPFEDHVKLVNEVTEFAKTCVADESAENCDKSLHTLFGDKLCTVATLRETYGEMADCCAKQEPERNECFLQHKDDNPNLPRLVRPEVDVMCTAFHDNEETFLKKYLYEIARRHPYFYAPELLFFAKRYKAAFTECCQAADKAACLLPKLDELRDEGKASSAKQRLKCASLQKFGERAFKAWAVARLSQRFPKAEFAEVSKLVTDLTKVHTECCHGDLLECADDRADLAKYICENQDSISSKLKECCEKPLLEKSHCIAEVENDEMPADLPSLAADFVESKDVCKNYAEAKDVFLGMFLYEYARRHPDYSVVLLLRLAKTYETTLEKCCAAADPHECYAKVFDEFKPLVEEPQNLIKQNCELFEQLGEYKFQNALLVRYTKKVPQVSTPTLVEVSRNLGKVGSKCCKHPEAKRMPCAEDYLSVVLNQLCVLHEKTPVSDRVTKCCTESLVNRRPCFSALEVDETYVPKEFNAETFTFHADICTLSEKERQIKKQTALVELVKHKPKATKEQLKAVMDDFAAFVEKCCKADDKETCFAEEGKKLVAASQAALGL

SEQ ID NO: 2 - DNA, 1758 bp, Homo sapiens
  source 1..1758: mol_type = other DNA; note = Nucleic Acid sequence of mature HSA
atggacgcacacaagagcgaggttgcccaccgtttcaaggacttaggagaggagaatttcaaggcattagtccttatcgcattcgcccaatacttacaacaatgtcccttcgaggaccacgttaagctcgtaaatgaggttacggagttcgccaagacgtgtgttgccgacgagagtgcagagaattgtgacaagtcattgcacacgttattcggtgacaagttgtgtacggttgccactcttcgtgagacatacggggagatggccgactgttgtgccaagcaagagccagagcgtaatgagtgtttcttacaacacaaggacgacaatccaaatttacctcgtctcgtccgtcctgaggttgacgtaatgtgtacggctttccacgacaatgaggagacgttcctcaagaagtacttgtacgagatcgcgcgccgtcacccatacttttacgctccagagttacttttcttcgcaaagcgttacaaggccgctttcactgagtgttgtcaagccgccgacaaggccgcctgtctcttacccaagcttgacgagttgcgtgacgaggggaaggcaagttccgcaaagcaacgtttaaagtgtgcttcactgcaaaagttcggagagcgtgccttcaaggcttgggcagttgcccgtttgtctcaacgtttcccaaaggcagagttcgcagaggtaagtaagcttgtcacggacttgacaaaggttcacacggagtgttgccacggagacctcttggagtgtgcagacgaccgtgcagaccttgcaaagtacatctgtgagaatcaagactcaatctcgtctaagttaaaggagtgttgtgaaaagcccttgcttgaaaagagtcactgtatcgcagaggtagagaatgacgagatgcccgctgacttaccctcattggccgcagacttcgtagagtcgaaggacgtttgtaagaattacgccgaggccaaggacgttttcttaggtatgttcttgtacgagtacgcacgtcgtcaccccgactactcggttgtccttctcttacgtttagctaagacgtacgagacgacattggaaaagtgttgtgccgctgccgaccctcacgagtgttacgctaaggtcttcgacgagttcaagccattggtagaggagccacaaaatttaatcaagcaaaattgtgagttattcgagcaactcggtgagtacaagttccaaaatgcactcctcgtacgttacacgaagaaggtaccccaagtctctacgccaactcttgttgaggtatcccgtaatcttgggaaggtcggaagtaagtgttgtaagcaccccgaggctaagcgtatgccttgtgcagaggactacttatcagtagtcctcaatcaattgtgtgttttgcacgaaaagacgccagtttccgaccgtgtcacaaagtgttgtacagagagtctcgttaatcgtcgtccctgtttcagtgcattggaagtcgacgagacgtacgttccaaaggagttcaatgcagagactttcacattccacgccgacatctgtactcttagtgaaaaggagcgtcaaatcaagaagcaaacagccttggtcgagcttgtcaagcacaagcccaaggccacgaaggagcaattaaaggccgtaatggacgacttcgcagccttcgtagaaaagtgttgtaaggccgacgacaaggagacttgtttcgccgaggaaggtaagaagcttgtagccgctagtcaagccgccttgggcctg

SEQ ID NO: 3 - protein, 586 aa, synthetic construct
  source 1..586: note = Albumin Synthetic variant
MDAHKSEVAHRFKDLGEENFKALVLIAFAQYLQQCPFEDLVKMVNEVTEFAKTCVADESAENCDKSLHTLFGDKLCTVATLRETYGEMADCCAKQEPERNECFLQHKDDNPNLPRLVRPEPDVMCTAFHDNEETFLKKYLYEIARRHPYFYAPELLYFAKRYKAAFTECCQAADKAACLLPKLDELREEGKASSAKQRHKCAILQKFGERAFKAWAVARLSQRFPKAEFAEVSKLVTDLTKVHTECCHGDLLECADDRADLAKYICENQDSISSKLKECCEKPLLEKSHCIAEVENDEMPADLPSLAADFIESKDVCKNYAEAKDVFLGMFLYEYARRHPDYSVVLLLRLAKTYETTLEKCCAAADPHECYSKVFDEFKPLIEEPQNLIKQNCELFEQLGEYKFQNALLIRYTKKVPQVSTPTLVEVARNLGKVGSKCCKHPEAKRMPCAEDYLSIVLNQLCVLHEKTPVSDRVTKCCTESLVNRRPCFSALEVDETYVPKEFNAETFTFHADICTLSEEERQIKKQTALVELVKHKPKATKEQLKAVMDDFSAFVEKCCKADDKETCFAEEGKKLIAASQAALGL

SEQ ID NO: 4 - DNA, 1758 bp, synthetic construct
  source 1..1758: mol_type = other DNA; note = Albumin Synthetic variant
atggatgcacataaaagcgaggtggcacatcgttttaaggatctgggcgaggagaactttaaagcactggtgttgattgctttcgctcagtatctccaacaatgcccgttcgaagacttggttaagatggtaaatgaagtcacagaatttgcgaaaacctgtgtggctgatgagtcggccgagaattgcgacaaaagtcttcacacgctgtttggtgacaaactgtgcactgttgctactctccgggaaacttatggcgaaatggcggactgttgcgcaaaacaagagccagagcgtaacgagtgtttcttacagcacaaagacgacaacccgaacctgccgcgcctcgtccgtccggaaccggatgtcatgtgtactgcgtttcatgacaatgaagaaacatttttgaaaaagtatctgtatgaaatcgctcgccgccacccgtacttttacgccccagagttgctctattttgctaaacgttacaaggccgcatttacggaatgttgtcaggcggctgataaagcggcttgtttgctgccgaaacttgatgagctgcgtgaggaagggaaagcttctagcgccaagcagcgtcataaatgtgccattctccagaagtttggcgaacgggccttcaaagcgtgggcagtcgcacgtctgagccaacgtttcccgaaggcggaatttgccgaagtcagcaaattggtgacagatctcactaaagttcacaccgagtgctgtcatggcgacctgcttgaatgcgcggatgaccgggccgacctggctaaatatatctgcgaaaaccaggattcaattagttccaaactgaaagaatgttgcgagaaacccttgctggagaaatcccattgcattgctgaagttgaaaatgatgagatgccggccgatttgccgagcctggcagctgatttcattgagtcaaaggacgtgtgcaagaactatgcagaagccaaagacgtttttctgggtatgttcctgtatgaatatgcccgccgtcatcccgactatagcgtcgtgctgttattgcgcctggccaagacttatgagacgaccctggagaaatgctgcgccgctgctgatcctcatgaatgctattccaaagtattcgacgagttcaaaccgttgatcgaagaaccgcaaaatcttattaaacaaaattgcgaattgtttgaacaactgggcgagtacaaatttcaaaatgctctcttaattcgttatactaagaaagtgccgcaagtctccacgcctacgctggtagaagtcgcccgtaacctgggtaaagtaggctctaaatgctgtaagcaccctgaggccaagcggatgccttgcgccgaagactacttgagcatcgtattgaatcagctctgtgtgttacacgagaaaaccccggtgtcagaccgtgtcacgaaatgttgtaccgagagccttgtgaaccgtcgtccatgcttctcagcactggaagttgacgaaacatacgtgccaaaagagtttaacgctgaaacttttacttttcatgcagacatctgcacgttgagcgaagaagaacgtcagattaaaaagcagactgcgctggtggagttagtgaaacataaacccaaagctactaaagaacagctcaaagcggtcatggacgacttcagcgcctttgttgagaaatgctgcaaggcggacgataaagagacctgttttgcggaagaaggtaagaaactgattgccgcaagccaggcagcactggggctg

SEQ ID NO: 5 - protein, 586 aa, synthetic construct
  source 1..586: note = Albumin Synthetic variant
MDAHKSEVAHRFKDLGEENFKALVLIAFAQYLQQCPFEDLVKMVNEVTEFAKTCVADESAENCDKSLHTLFGDKLCTVATLRETYGEMADCCAKQEPERNECFLQHKDDNPNLPRLVRPEPDVMCTAFHDNEETFLNKYLYEIARRHPYFYAPELLYFAKRYKAAFTECCQAADKAACLLPKLDELREEGKASSAKQRHKCAILQKFGERAFKAWAIARLSQRFPKAEFAEVSKLVTDLTKVHTECCHGDLLECMDDRADLAKYICENQDSISSKLKECCEKPLLEKSHCIAEVENDEMPADLPSLAADFIESKDVCKNYAEAKDVFLGMFLYEYARRHPDYSVTLLLRLAKTYETTLEKCCAAADPHECYSKVFDEFKPLIEEPQNLIKQNCELFEQLGEYKFQNALLIRYTKKVPQVSTPTLVEVARNLGKVGSKCCKLPEAKRMPCIEDYLSIVLNQLCVLHEKTPVNDRVTKCCTESLVNRRPCFSALEVDETYVPKEFNAETFTFHADICTLSEEERQIKKQTFLVELVKHKPKATKEQLKAIMDDFSAFVEKCCKADDKETCFAEEGKKLIAASQAALGL

SEQ ID NO: 6 - DNA, 1758 bp, synthetic construct
  source 1..1758: mol_type = other DNA; note = Albumin Synthetic variant
atggatgcacataaaagcgaggtggcacatcgttttaaagatctgggcgaagaaaattttaaagcgttagtgttgatcgcgttcgctcagtatttacaacaatgcccgttcgaggatttggtcaaaatggttaacgaagtaacagagtttgcaaaaacctgtgtcgccgatgagtcagcagagaactgcgataaaagcctgcacacgcttttcggcgataaactgtgcactgtggctacactccgcgaaacgtatggtgaaatggccgattgttgcgcgaaacaggagccggaacgcaatgaatgttttttgcagcataaagatgataatccaaatctcccacggctcgttcgcccggagcctgatgttatgtgtaccgcattccacgacaatgaagaaacgtttctcaataagtacctgtatgagattgctcgtcgtcatccatacttttacgctccggaattactgtacttcgctaagcgttacaaggcagcctttacagagtgctgtcaagcggcagacaaagcggcctgcttgcttccgaaacttgacgaacttcgcgaagaagggaaagcctcgtccgccaaacaacggcacaaatgtgccattctccagaagtttggtgagcgcgcatttaaagcgtgggccattgcgcggctgtcacagcgtttcccgaaagcggaatttgcggaagtgagtaaactggtgactgatttgacgaaagtgcataccgaatgttgtcatggcgatttgttggaatgcatggatgatcgtgcagatttagccaaatatatttgcgaaaatcaggatagcatttctagcaagctgaaagaatgttgtgagaaacctctgctggagaaatctcattgcatcgcggaggttgaaaatgatgaaatgccggcggatctgcctagtctggcagcggatttcattgaaagcaaagatgtctgcaagaattatgcggaagcgaaagatgtatttttaggtatgtttctttacgagtatgctcgccgtcacccggattacagtgtcaccctgttgctgcgcttagccaaaacgtatgaaaccacgctggaaaagtgttgcgccgcggcggaccctcacgaatgttattcgaaagtttttgatgagtttaaacctcttatcgaggagccccaaaatctcattaaacaaaactgcgaactgtttgagcaactgggggaatacaaattccagaacgctttattgattcgctatactaagaaagtgccccaagtgtcaacgccgacgctggtagaagttgcccgcaacttagggaaggtgggcagcaaatgctgtaaacttccagaagctaagcgtatgccatgtatcgaagattatctgtccattgttctgaatcagttatgtgtgctccatgaaaaaacccctgtcaatgatcgggttaccaagtgctgcacggaatccctcgtcaatcgtcgcccatgctttagcgcccttgaagtagacgaaacatacgtcccgaaagagttcaatgccgaaacgtttacctttcatgcagacatttgcaccctcagcgaggaagaacgccaaatcaaaaagcagaccttccttgtggaacttgtgaagcataaaccaaaagcgacgaaagaacagctgaaagcgattatggatgatttcagtgcctttgtagaaaagtgctgtaaagccgacgacaaagaaacatgctttgcggaggagggcaagaagctcattgccgcaagccaggcagcactggggctg

SEQ ID NO: 7 - protein, 586 aa, synthetic construct
  source 1..586: note = Albumin Synthetic variant
MDAHKSEVAHRFKDLGEENFKALVLIAFAQYLQKCPFEELVKMVKEVTEFAKKCVADETAENCDKSLHTLFGDKLCQVATLRETYGEMADCCAKQDPERHECFLQHKDDNPNLPRLERPEVDVMCKAFHDNEETFLNKYLYEIARRHPYFYAPELLYFAKRYKKAFTECCQAEDKAACLLPKLDALREEGKESSAKQRYKCAILQKFGERVFKAWAIARLSQRFPKAPFEEISKLVTDLTKVHKACCHGDMLECMDDRAKLAKYICENQDSISSKLKECCEKPLLERSHCIAEVENDDKPEDLPPLAADFVESKDVCKNYAEAKDVFLARFLYEYARRHPDYSVTLLLRIAKTYEDTLEKCCKAEDPHECYAKVEEEFKKLVEETQNLIKQNCELFEKLGEYYFQNALLIRYTKKMPQVPTDTLVELTRNLGKVGSKCCKLPEEKRLPCIEDYLSIVLNQLCVLHEKTPVNDRVTKCCTESLVNRRHCFSALEVDETYVPKEFNAETFTFHADLCTLSEEERQIMKQKFLVELVKHKPKATEEQLKAVMDDFTAFVEKCCKAEDPETCFAEEGSKLIAKSQAALGL

SEQ ID NO: 8 - DNA, 1758 bp, synthetic construct
  source 1..1758: mol_type = other DNA; note = Albumin Synthetic variant
atggatgcacataaaagcgaggtggcacatcgttttaaagatttaggtgaagaaaactttaaagctctcgttctgatcgcgtttgcccagtaccttcagaaatgcccgttcgaagagctcgttaaaatggtcaaagaggtaacggagttcgcgaagaaatgcgtagcagatgaaactgcggaaaactgtgataagtctttacacactctttttggagataagttatgccaagttgccacgctgcgtgagacgtacggtgagatggcggattgctgcgcaaaacaagatccggagcgtcacgaatgctttttgcagcacaaagatgacaacccaaatttaccgcgtttggagcgtccggaagtggatgttatgtgtaaagccttccacgataacgaagagacgtttttaaataaatacctgtacgaaattgcgcggcgtcatccatatttctatgcgccggagcttctgtattttgccaaacgttacaagaaggcttttactgaatgctgccaggcggaagataaagccgcgtgcttgctccctaagctggatgccttgcgtgaggaaggtaaagaatcttcggccaaacagcgctataaatgcgcgatcctccagaaatttggagagcgcgtctttaaagcgtgggccattgcgcggctttcacagcgttttcctaaagcgccgtttgaagagatctcgaaactggttaccgatctgacaaaagttcacaaagcttgctgtcatggtgatatgctggaatgcatggacgatcgtgcgaaactcgcgaaatatatttgcgaaaatcaggattcgattagttccaagcttaaagaatgctgcgagaaaccgctgttggaacgcagtcactgtattgcggaagtggagaacgatgataaaccggaggatctgccgccattagccgcagattttgtggagagcaaagacgtctgcaagaattatgccgaggcaaaggatgtctttctggctcgtttcttatacgaatatgcgcgtcggcacccggattactccgttaccctcttattgcgtattgccaaaacgtatgaagataccctggagaagtgctgcaaggcggaagatcctcatgaatgttacgcgaaagtcgaggaggaatttaaaaagctggtagaagaaacgcaaaacttaatcaagcaaaattgcgaattatttgagaaactgggtgaatattattttcaaaacgccctgctcattcgctatactaagaaaatgccgcaggtcccaacggacacgctcgtcgaattgacccggaacttaggcaaagtgggatcgaaatgctgtaaacttccggaagagaaacgcctgccgtgcatcgaagattacctctctatcgtgctcaaccagctgtgtgttctgcatgagaagaccccggtgaatgatcgtgttaccaagtgctgtacggaatcactggttaatcgtcgccattgctttagtgccctggaagtcgatgaaacttatgtcccaaaagagttcaacgccgaaacatttacctttcatgcggatttgtgcaccctttccgaagaagaacgtcagatcatgaaacagaaatttcttgtcgagctggtcaaacacaaaccgaaagccaccgaagaacagctgaaagcagttatggacgatttcaccgcctttgttgagaaatgctgtaaagcagaagatcctgaaacctgctttgcggaagaaggttcgaaactgattgccgcaagccaggcagcactggggctg

SEQ ID NO: 9 - protein, 584 aa, Bos taurus
  source 1..584: note = Amino Acid sequence of mature BSA
MDTHKSEIAHRFKDLGEEHFKGLVLIAFSQYLQQCPFDEHVKLVNELTEFAKTCVADESHAGCEKSLHTLFGDELCKVASLRETYGDMADCCEKQEPERNECFLSHKDDSPDLPKLKPDPNTLCDEFKADEKKFWGKYLYEIARRHPYFYAPELLYYANKYNGVFQECCQAEDKGACLLPKIETMREKVLTSSARQRLRCASIQKFGERALKAWSVARLSQKFPKAEFVEVTKLVTDLTKVHKECCHGDLLECADDRADLAKYICDNQDTISSKLKECCDKPLLEKSHCIAEVEKDAIPENLPPLTADFAEDKDVCKNYQEAKDAFLGSFLYEYSRRHPEYAVSVLLRLAKEYEATLEECCAKDDPHACYSTVFDKLKHLVDEPQNLIKQNCDQFEKLGEYGFQNALIVRYTRKVPQVSTPTLVEVSRSLGKVGTRCCTKPESERMPCTEDYLSLILNRLCVLHEKTPVSEKVTKCCTESLVNRRPCFSALTPDETYVPKAFDEKLFTFHADICTLPDTEKQIKKQTALVELLKHKPKATEEQLKTVMENFVAFVDKCCAADDKEACFAVEGPKLVVSTQTALA

SEQ ID NO: 10 - DNA, 1752 bp, Bos taurus
  source 1..1752: mol_type = other DNA; note = Nucleic Acid sequence of mature BSA
atggatacccataagagtgaaattgcccatcgatttaaggacctcggtgaagaacactttaaggggcttgtgttaatagcattctcgcagtatcttcagcaatgtccgtttgatgaacacgttaaattagtgaacgaattaactgagttcgccaaaacgtgcgtagcggacgaaagtcatgcgggatgcgagaagagccttcatacgctgtttggtgacgaactgtgcaaggtggcgagtctgcgtgaaacgtacggggacatggctgattgctgcgaaaaacaggaaccggaacgcaacgagtgcttcctgtctcataaagatgattccccggatcttcccaaattgaaacctgaccccaatacattgtgcgatgaatttaaggctgatgaaaagaaattttggggcaagtatctgtatgaaatcgcgcggagacatccttatttctacgcaccggaactgctgtactacgcgaacaagtataatggggtatttcaggaatgttgccaggcagaagataaaggagcctgcctgctccccaaaattgaaactatgcgtgagaaggtgctgacatctagcgcacggcaacgtttacgatgcgcgtcaatacaaaaatttggagaacgcgctcttaaagcttggtctgttgcacgtctgtcacagaaatttccaaaagccgagtttgtcgaagttaccaagctggtgacggatcttacgaaggtacataaggagtgctgtcacggcgatctgctggagtgtgcagatgatagagctgaccttgcaaagtacatttgcgacaatcaagataccataagttcgaagcttaaagagtgttgcgacaaaccgctgcttgaaaaaagccattgtatcgcagaggtcgaaaaagatgctatccccgaaaacttaccgccactgaccgcggacttcgcagaggacaaagatgtttgtaaaaattatcaggaggccaaagatgcatttcttgggtcctttttgtatgagtattcacggcgacatccagaatacgctgtctctgtcctgctccggctggctaaagaatatgaagcaactttagaagaatgttgcgccaaagatgatccgcatgcttgttacagtacggtgtttgataaactgaaacacctcgtggatgaacctcagaacttgataaagcaaaattgcgatcagttcgaaaaattaggtgagtacgggttccagaatgcactgatcgttcggtatacgcgtaaagttccgcaagttagcactccaactctggttgaggtatcccgcagtctcggtaaagtcggaactcgctgttgcactaaaccggaaagtgagagaatgccgtgtactgaagattacctgagtctgattcttaatcggttatgcgtgctgcatgaaaagacccctgtgagtgagaaagttaccaaatgttgtactgaatccctggtcaaccgccgtccgtgctttagcgcactcaccccagatgaaacttatgtgcctaaggcattcgatgagaaactgtttacctttcatgcagatatctgtaccctgcctgatactgagaaacagattaagaaacagacagctctggtggaactcctgaaacataagccaaaagccacggaggaacagcttaaaaccgttatggagaatttcgtggcttttgtcgataagtgttgtgcggcggatgataaagaggcgtgctttgccgttgaaggtcctaaacttgtagtctcaacccaaacagcgctggca

SEQ ID NO: 11 - protein, 584 aa, synthetic construct
  source 1..584: note = Albumin Synthetic variant
MDTHKSEIAHRFKDLGEEHFKALVLIAFAQYLQQCPFDELVKMVNELTEFAKTCVADESHAGCEKSLHTLFGDELCKVASLRETYGDMADCCEKQEPERNECFLSHKDDSPDLPKLKPDPNTLCDEFKADEKKFWGKYIYEIARRHPYFYAPELLYYANKYNGIFQECCQAEDKAACLLPKIETIREKVLTSSARQRLRCASLQKFGERALKAWSVARLSQKFPKAEFVEITKLVTDLTKVHKECCHGDLLECADDRADLAKYICDNQDTISSKLKECCDKPLLEKSHCIAEVEKDAIPENLPPLTADFLEDKDVCKNYQEAKDAFLGSFLYEYSRRHPEYAVSVLLRLAKEYEATLEECCAKDDPHACYSTVFDKLKHLIDEPQNLIKQNCDQFEKLGEYGFQNALIIRYTRKVPQVSTPTLVEVTRSLGKVGTRCCTKPESERMPCTEDYLSLILNRLCVLHEKTPVSEKVTKCCTESLVNRRPCFSALTPDETYVPKAFDEKLFTFHADICTLPDEEKQIKKQTALVELLKHKPKATEEQLKTVMENFVAFVDKCCAADDKEACFAVEGPKLIVSTQTALA

SEQ ID NO: 12 - DNA, 1752 bp, synthetic construct
  source 1..1752: mol_type = other DNA; note = Albumin Synthetic variant
atggatacccataagagtgaaattgcccatcgttttaaggatttaggcgaggaacattttaaagctctcgtgctgattgcctttgcacaataccttcagcaatgtccattcgatgaactggttaagatggttaatgaacttaccgagttcgcaaagacgtgtgtggcggatgaatctcacgcaggttgcgaaaaaagcctgcatactctttttggtgatgaattgtgtaaagtagcaagccttcgtgaaacctatggtgatatggcagattgttgcgaaaaacaagaaccggagagaaatgaatgtttcttgagtcataaggacgattcaccggatctgccgaagttgaaacctgacccaaataccctttgcgatgaatttaaagccgatgaaaaaaaattctgggggaaatatatctatgaaattgctagacgccatccttatttttatgcgccagaattgttgtactacgcaaataaatacaacgggatattccaggagtgttgtcaggcagaagataaggccgcctgtctcctgcctaaaatcgagactataagagaaaaggtcttgacttcttctgctcgtcagagactgagatgtgcaagtcttcagaaatttggggaaagagcactgaaagcctggagtgttgcacgattaagccagaaatttcctaaagccgagtttgttgagatcacgaaacttgtcactgaccttacgaaagttcataaagaatgttgccacggagatctgctggaatgtgcggatgatcgtgccgatcttgctaaatatatctgtgataaccaagatacaatctcttcaaagctgaaagaatgttgtgacaaacctttgttagagaaatcacattgtattgccgaagttgagaaagatgccataccggaaaacctcccaccgttgaccgcagactttctggaggataaggacgtatgcaaaaattaccaggaagctaaggatgcgttcctgggtagcttcctgtatgaatattcacgccgccaccccgagtatgcggtctcagtgctgttacgcttagcgaaagaatacgaggccacgctggaagaatgctgcgcaaaagatgacccacatgcctgttactctacggtatttgataaacttaaacaccttattgatgaacctcagaacttaatcaaacaaaattgtgaccagtttgagaagctcggtgaatatggttttcaaaatgcactcataattcgctatacccgcaaggtcccacaggtctccacgccgacactggtagaagtgacccgttcgctcggcaaggtaggaacgcgttgttgtacgaaacctgaaagtgaacgtatgccttgcacagaagactatctgtcgctgattctcaatcgtttatgcgtactgcatgaaaagacaccagtctcggaaaaagtgacaaagtgctgcacggagtcattggtcaaccgtagaccatgttttagcgcccttacaccggatgaaacttatgtaccgaaagctttcgatgagaaattattcaccttccatgcggatatctgcaccctgcctgatgaagagaagcagatcaagaaacagacagccttagtcgagttattaaagcacaaacctaaagcgacggaagagcaactgaaaacagtaatggaaaactttgtggccttcgtcgataaatgttgcgccgcagatgataaagaagcatgttttgccgttgaaggtccgaagttaattgttagtacccaaaccgcattagca

SEQ ID NO: 13 - protein, 584 aa, synthetic construct
  source 1..584: note = Albumin Synthetic variant
MDTHKSEIAHRFKDLGEEHFKALVLIAFAQYLQQCPFDELVKMVNELTEFAKTCVADESHAGCEKSLHTLFGDELCKVASLRETYGDMADCCEKQEPERNECFLSHKDDSPDLPKLKPDPNTLCDEFKADEKKFWGKYIYEIARRHPYFYAPELLYYANKYNGIFQECCQAEDKAACLLPKIETIREKVLTSSARQRLRCASLQKFGERALKAWSVARLSQKFPKAEFVEITKLVTDLTKIYKECCHGDLLECMDDRADLVKYICDNQDTISSKLKECCDKPLLEKSHCIAEVEKDAIPENLPPLTADFLEDKDVCKNYQEAKDAFLGSFLYEYSRRHPEYAVSLLLRLAKEYEATLEECCAKDDPHACYSTVFDKLKHLIDEPQNLIKQNCDQFEKLGEYGFQNALIIRYTRKMPQVSTPTLVEITRSLGKVGTRCCTLPESERLPCTEDYLSLILNRLCVLHEKTPVSEKVTKCCTESLVNRRHCFSALTPDETYVPKAFDEKLFTFHADICTLPDEEKQIKKQTFLVELLKHKPKATEEQLKTIMENFTAFVDKCCAADDKEACFAVEGPKLIVSTQTALA

SEQ ID NO: 14 - DNA, 1752 bp, synthetic construct
  source 1..1752: mol_type = other DNA; note = Albumin Synthetic variant
atggatacccataagagtgaaattgcccatcgctttaaagatctcggggaggagcactttaaagcccttgtcctgatcgccttcgcacagtatctgcaacagtgcccttttgatgaattggtcaagatggttaatgaattaaccgagttcgctaaaacttgcgtcgctgatgagtctcacgcaggatgcgagaaatcactgcatacattgttcggtgatgaattgtgcaaggtcgctagcttgcgtgaaacctacggcgatatggccgattgctgtgaaaaacaggagccggagcgtaatgagtgtttcttaagtcacaaggatgattctccagatcttccaaagttaaaaccagatccaaatactctttgtgatgagttcaaagcggatgaaaagaaattttggggtaaatacatctacgagattgcccgtcggcatccctacttctatgccccggaactgctgtactatgcgaataagtataacggaattttccaggaatgttgtcaagctgaagataaagccgcttgtctgctgcctaaaattgagacaattcgggaaaaagtactgacgagctccgcacgtcaacgcctgcgatgcgcgagtctgcaaaagtttggtgaacgtgctcttaaagcctggagcgtcgcgcgactctcacagaaatttccaaaagcagagtttgtcgaaattaccaaacttgtcactgacctgaccaagatatataaggaatgctgccacggcgatttgctggagtgcatggatgatcgggccgacttagtgaaatatatatgtgacaaccaagataccatatcaagcaagctgaaagagtgttgtgataagccgttgctcgaaaagtcgcactgcattgcggaggtcgaaaaagacgctatccctgaaaacttaccgccgttaacagccgattttcttgaagacaaagacgtttgcaaaaactatcaggaagccaaagatgcatttctcggcagtttcttatatgagtactccagacgccacccggaatatgcagtttcgcttctcttaagacttgcaaaagaatacgaggccaccctggaggagtgctgtgctaaagatgacccacatgcatgttattctaccgtgtttgacaaactgaagcatcttatcgacgagccccagaatctgatcaaacagaattgcgaccaattcgagaaattaggtgagtatggtttccaaaacgcgctcatcatccgatacacccgcaagatgccgcaagtctcaacccctacactggtggagatcacccgcagcctgggtaaagtgggtacacgatgctgtaccctcccggaaagcgaacgtcttccttgtacagaagactacttatcgctcatattaaaccgtctgtgcgttttgcacgaaaagacccctgtttcggagaaggtgaccaaatgttgcactgaaagtctggttaatcggcggcattgcttctctgcgctgacacctgatgaaacctatgtaccaaaagcctttgatgaaaagttatttacgtttcacgccgacatttgcacactgccggatgaggaaaaacagatcaagaaacaaacttttctggtagaactgctgaaacataagccgaaagcaacggaagaacagttaaaaaccattatggagaactttaccgcgttcgtggataagtgctgtgccgcagacgataaagaagcctgttttgcagtggagggaccgaaactgatagttagcacccaaaccgcgctcgcg

SEQ ID NO: 15 - protein, 584 aa, synthetic construct
  source 1..584: note = Albumin Synthetic variant
MDTHKSEIAHRFKDLGEEHFKALVLIAFAQYLQKCPFDELVKMVNDLTEFAKKCVADESHPGCSKSLHTLFGDELCKVEELRETYGDMADCCSKQEPERNECFLSHKDDNPDLPKLKPDPNTLCKEFKEDEKKFWGKYIYEIARRHPYFYAPELLYYAKKYNKIFQECCQAEDKAACLLPKIEAIREKVKTSSARQRLRCASLQKFGERALKAWFVARLSQKFPKAPFEEITKLVTDLTKIYKECCHGDLLECMDDRAKLVKYICDNQDTISSKLKECCDKPLLERSHCIAEVEDDDIPEDLPPLVADFLEDKDVCKNYQEDKDAFLGRFLYEYSRRHPEYAVSLLLRLAKEYEATLEECCKKDDPHACYSRVFEKLKKHIDEPQELIKQNCDQFEKLGEYGFQNALIIRYTKKMPQVPTDTLVEITRSLGKVGTRCCQLPEEKRLPCTEDYLSLILNRLCVLHEKTPVSEKVTKCCTESLVNRRHCFSALTPDETYVPKPFDPKLFTFHADICTLPPEEKQIKKQKFLVELLKHKPKATEEQLKTIMENFTAMVDKCCKAEDKEACFAEEGPKLIEKTQAALA

SEQ ID NO: 16 - DNA, 1752 bp, synthetic construct
  source 1..1752: mol_type = other DNA; note = Albumin Synthetic variant
atggatacccataagagtgaaattgcccatcgtttcaaagaccttggagaagaacactttaaagctctcgtgctcattgccttcgcgcaatatctccaaaagtgtccttttgatgagttggtaaagatggtaaacgatttgacagagtttgcgaagaaatgtgttgcggatgaatcgcatccaggttgcagtaagagcctgcacactctgtttggagatgaactttgtaaagtagaggaactgcgagaaacctacggagatatggctgactgttgcagcaaacaggagcctgaacggaatgaatgcttcctctcccataaggacgacaatcccgacttgccgaaattgaagcccgatccgaacactctgtgcaaagaatttaaagaagatgaaaagaaattttggggcaaatacatttatgaaatagcccgccggcatccgtatttctatgccccggaattactttattatgcgaagaaatataacaaaatctttcaagaatgctgccaggctgaagataaagcagcttgcttgctcccgaaaattgaagcgattcgggaaaaagtgaaaacttcttcagctcgccagcgtctgcgttgtgcttcattacagaaatttggcgaacgggctctgaaagcctggtttgtcgcacgtctgtcacagaagtttcccaaggctccgtttgaggaaattacgaagttggtcacagacttaacaaaaatttataaagaatgttgtcacggtgatctgctggaatgtatggatgatcgtgccaagctggtaaagtacatttgtgataatcaagatacgataagttcaaagttaaaggagtgttgcgataaaccacttttagagagaagtcactgtattgcggaagtcgaggatgatgatatcccggaggacctccctcctcttgtagcggattttctggaggataaagatgtctgtaaaaattatcaggaagataaagacgcttttcttggccgttttttatacgaatatagcagacgtcaccccgaatatgctgtgtctttgttgcttcgccttgcaaaggagtacgaagcaactctggaggaatgctgtaaaaaagacgatccacacgcttgttatagtcgggtctttgagaaactgaagaaacatatagatgagccgcaagaactgataaaacagaactgcgaccagtttgagaagctgggggaatacggcttccaaaatgcattgataattagatacactaaaaagatgccgcaagtgccgacggataccctcgttgagataactcggagtttaggaaaagtaggcacacggtgttgccagcttccggaagaaaaacgcttgccttgcactgaggactatttatccctcattttaaaccggctgtgcgtacttcatgaaaagactccagtgagtgagaaggttaccaaatgttgcactgaaagcctggtgaatagacgtcactgtttttcagcgttaactccagatgaaacttatgtccccaaaccttttgatcctaaattgttcacctttcacgctgatatatgtaccttacctcccgaagaaaaacagatcaagaagcagaaatttttggtggaacttttgaaacataagccgaaagctaccgaagaacagttgaaaactattatggaaaactttacagctatggtcgataagtgttgtaaagctgaggataaagaagcttgttttgccgaagagggaccaaaactgattgagaaaacccaagcggccctggct

SEQ ID NO: 17 - protein, 585 aa, synthetic construct
  source 1..585: note = Design 7 - raw design of HSA
DAHKSEVAHRFKDLGEENFKALVLIAFAQYLQKCPFEELVKMVKEVTEFAKKCVADETAENCDKSLHTLFGDKLCQVATLRETYGEMADCCAKQDPERHECFLQHKDDNPNLPRLERPEVDVMCKAFHDNEETFLNKYLYEIARRHPYFYAPELLYFAKRYKKAFTECCQAEDKAACLLPKLDALREEGKESSAKQRYKCAILQKFGERVFKAWAIARLSQRFPKAPFEEISKLVTDLTKVHKACCHGDMLECMDDRAKLAKYICENQDSISSKLKECCEKPLLERSHCIAEVENDDKPEDLPPLAADFVESKDVCKNYAEAKDVFLARFLYEYARRHPDYSVTLLLRIAKTYEDTLEKCCKAEDPHECYAKVEEEFKKLVEETQNLIKQNCELFEKLGEYYFQNALLIRYTKKMPQVPTDTLVELTRNLGKVGSKCCKLPEEKRLPCIEDYLSIVLNQLCVLHEKTPVNDRVTKCCTESLVNRRHCFSALEVDETYVPKEFNAETFTFHADLCTLSEEERQIMKQKFLVELVKHKPKATEEQLKAVMDDFTAFVEKCCKAEDPETCFAEEGSKLIAKSQAALGL

SEQ ID NO: 18 - protein, 583 aa, synthetic construct
  source 1..583: note = Design 6 - raw design of BSA
DTHKSEIAHRFKDLGEEHFKGLVLIAFAQYLQKCPFDELVKLVNDLTEFAKKCVADESHPGCSKSLHTLFGDEICKVEELRETYGDMADCCSKQEPERNECFLSHKDDNPDLPKLKPDPNTLCKEFKEDEKKFWGKYIYEIARRHPYFYAPELLYYAAKYNKVFQECCQAEDKAACLLPKIEAIREKVKTSSARQRLRCASLQKFGERALKAWFVARLSQKFPKAPFEEITKLVTDLTKIYKECCHGDLLECMDDRAKLVKYICDNQDTISSKLKECCDKPLLERSHCIAELEFDDIPEDLPPLVADFLEDKDVCKNYQEDKDAFLGRFLYEYSRRHPEYAVSLLLRLAKVYEATLEECCKKDDPHACYSRVFEKLKKHIDEPQNLVKQNCDQFEKLGEYGFQNALIIRYTKKMPQVPTDTLVEVSRSLGKVGTRCCQLPEEKRLPCTEDYLSLILNRLCVLHEKTPVSEKVTKCCTESLVNRRHCFSALTPDETYVPKPFDPKLFTFHADICTLPPEELQIKKQKFLVELLKHKPKATEEQLKTVMENFTAMVDKCCKAEDKEACFAEEGPKLIEKTQAALA